European Patent Application EP 4 382 620 A2, published June 12, 2024. Title: COMPOSITIONS AND METHODS FOR DETECTING GASTROINTESTINAL PATHOGENS. Applicant: GEN-PROBE INCORPORATED. The sequence listing filed with the application follows.

SEQUENCE LISTING (49 sequences)

SEQ ID NO: 1 - DNA, 26 bp, synthetic construct
  misc_feature 1..26: note = Synthetic: E. coli Set1-stx1-Probe2
  misc_feature 1..26: note = none, one or more, or each of nucleotides 6, 7, 9, 14, 17, and 24 comprises 5-methylcytosine
  source 1..26: mol_type = other DNA
ctataccacgttacagcgtgttgcag

SEQ ID NO: 2 - DNA, 26 bp, synthetic construct
  misc_feature 1..26: note = Synthetic: E. coli Set1-stx1-Probe3
  misc_feature 1..26: note = none, one or more, or each of nucleotides 5, 8, 11, 13, 18, and 21 comprises 5-methylcytosine
  source 1..26: mol_type = other DNA
ttatctgcatccccgtacgactgatc

SEQ ID NO: 3 - DNA, 20 bp, synthetic construct
  misc_feature 1..20: note = Synthetic: E. coli Set1-stx1-RP2
  source 1..20: mol_type = other DNA
gaagtagtcaacgaatggcg

SEQ ID NO: 4 - DNA, 24 bp, synthetic construct
  misc_feature 1..24: note = Synthetic: E. coli Set1-stx2-FP2
  source 1..24: mol_type = other DNA
ccatgacaacggacagcagttata

SEQ ID NO: 5 - DNA, 23 bp, synthetic construct
  misc_feature 1..23: note = Synthetic: E. coli Set1-stx2-Probe4
  source 1..23: mol_type = other DNA
actctgcaacgtgtcgcagcgct

SEQ ID NO: 6 - DNA, 27 bp, synthetic construct
  misc_feature 1..27: note = Synthetic: E. coli Set1-stx2-Probe7
  misc_feature 1..27: note = none, one or more, or each of nucleotides 3, 7, 8, 15, 20, 24, and 27 comprises 5-methylcytosine
  source 1..27: mol_type = other DNA
aacgttccggaatgcaaatcagtcgtc

SEQ ID NO: 7 - DNA, 25 bp, synthetic construct
  misc_feature 1..25: note = Synthetic: E. coli Set1-stx2-RP
  misc_feature 1..25: note = none, one or more, or each of nucleotides 3, 4, 18, and 19 comprises 5-methylcytosine
  source 1..25: mol_type = other DNA
cgccagatatgatgaaaccagtgag

SEQ ID NO: 8 - DNA, 20 bp, synthetic construct
  misc_feature 1..20: note = Synthetic: C. coli Set1-cadF-FP
  source 1..20: mol_type = other DNA
gagcgtggcttatcttgacc

SEQ ID NO: 9 - DNA, 30 bp, synthetic construct
  misc_feature 1..30: note = Synthetic: C. coli Set1-cadF-Probe7
  misc_feature 1..30: note = none, one or more, or each of nucleotides 2, 6, 13, 16, 23, 26, 28, and 29 comprises 5-methylcytosine
  source 1..30: mol_type = other DNA
actgtctggatacgacttttatctacaccg

SEQ ID NO: 10 - DNA, 22 bp, synthetic construct
  misc_feature 1..22: note = Synthetic: C. coli Set1-cadF-RP
  source 1..22: mol_type = other DNA
cagaaagacgcgctaacagcgt

SEQ ID NO: 11 - DNA, 24 bp, synthetic construct
  misc_feature 1..24: note = Synthetic: C. jejuni Set1-glyA-FP3
  source 1..24: mol_type = other DNA
gctaatgttcagcctaattcaggt

SEQ ID NO: 12 - DNA, 21 bp, synthetic construct
  misc_feature 1..21: note = Synthetic: Salmonella Set1-InvA-FP
  misc_feature 1..21: note = none, one or more, or each of nucleotides 4, 11, 12, and 16 comprises 5-methylcytosine
  source 1..21: mol_type = other DNA
gaacgtgtttccgtgcgtaat

SEQ ID NO: 13 - DNA, 23 bp, synthetic construct
  misc_feature 1..23: note = Synthetic: Salmonella Set1-InvA-Probe6
  source 1..23: mol_type = other DNA
atggaagcgctcgcattgtgggc

SEQ ID NO: 14 - DNA, 29 bp, synthetic construct
  misc_feature 1..29: note = Synthetic: Salmonella Set1-InvA-RP3
  source 1..29: mol_type = other DNA
atataacgcgccattgcyccacgaatatg

SEQ ID NO: 15 - DNA, 24 bp, synthetic construct
  misc_feature 1..24: note = Synthetic: Shigella Set2-ipaH-FP
  misc_feature 3: note = n is inosine
  misc_feature 1..24: note = none, one or more, or each of nucleotides 7 and 15 comprises 5-methylcytosine
  source 1..24: mol_type = other DNA
agngtactcattctccagcatctc

SEQ ID NO: 16 - DNA, 23 bp, synthetic construct
  misc_feature 1..23: note = Synthetic: Shigella Set2-ipaH-Probe
  misc_feature 16: note = n is inosine
  source 1..23: mol_type = other DNA
ttctgctcttctgccngcgccca

SEQ ID NO: 17 - DNA, 20 bp, synthetic construct
  misc_feature 1..20: note = Synthetic: Shigella Set2-ipaH-RP
  source 1..20: mol_type = other DNA
tacggactggttctccctct

SEQ ID NO: 18 - DNA, 29 bp, synthetic construct
  misc_feature 1..29: note = Synthetic: C. jejuni Set1-glyA-Probe9
  misc_feature 1..29: note = none, one or more, or each of nucleotides 7 and 12 or none, one or more, or each of nucleotides 7, 12, and 25 comprises 5-methylcytosine
  source 1..29: mol_type = other DNA
ctcaagcyaatcaaggtgtttatgcggct

SEQ ID NO: 19 - DNA, 25 bp, synthetic construct
  misc_feature 1..25: note = Synthetic: C. jejuni Set1-glyA-RP2
  misc_feature 23: note = n is inosine
  misc_feature 1..25: note = none, one or more, or each of nucleotides 1, 2, 7, 14, 15, 19, and 20 comprises 5-methylcytosine
  source 1..25: mol_type = other DNA
ccatgacttaaatccattcctanaa

SEQ ID NO: 20 - DNA, 24 bp, synthetic construct
  misc_feature 1..24: note = Synthetic: E. coli Set1-stx1-FP2
  source 1..24: mol_type = other DNA
ggttacattgtctggtgacagtag

SEQ ID NO: 21 - DNA, 25 bp, synthetic construct
  misc_feature 1..25: note = Synthetic: Salmonella Set1-OrgC-FP
  misc_feature 14: note = n is inosine
  misc_feature 23: note = n is inosine
  misc_feature 1..25: note = none, one or more, or each of nucleotides 13, 17, and 24 comprises 5-methylcytosine
  source 1..25: mol_type = other DNA
aagagatgaatgcnttcaaagancc

SEQ ID NO: 22 - DNA, 23 bp, synthetic construct
  misc_feature 1..23: note = Synthetic: Shigella Set1-ipaH-RP
  misc_feature 1..23: note = none, one or more, or each of nucleotides 5 and 16 comprises 5-methylcytosine
  source 1..23: mol_type = other DNA
aatgcgtttctatggcgtgtcgg

SEQ ID NO: 23 - DNA, 26 bp, synthetic construct
  misc_feature 1..26: note = Synthetic: Salmonella Set2-InvA-Probe
  misc_feature 15: note = n is inosine
  misc_feature 1..26: note = none, one or more, or each of nucleotides 2, 5, 7, and 14 comprises 5-methylcytosine
  source 1..26: mol_type = other DNA
actgctcgtaattcnccgccattggc

SEQ ID NO: 24 - DNA, 25 bp, synthetic construct
  misc_feature 1..25: note = Synthetic: Shigella Set3-ipaH-Probe
  source 1..25: mol_type = other DNA
agggagagcagagcgccggtatcat

SEQ ID NO: 25 - DNA, 20 bp, synthetic construct
  misc_feature 1..20: note = Synthetic: Salmonella Set2-OrgC-Probe3
  misc_feature 5: note = n is inosine
  misc_feature 8: note = n is inosine
  misc_feature 1..20: note = none, one or more, or each of nucleotides 7, 9, 13, and 15 comprises 5-methylcytosine
  source 1..20: mol_type = other DNA
tgaangcncagtcacaaatg

SEQ ID NO: 26 - DNA, 24 bp, synthetic construct
  misc_feature 1..24: note = Synthetic: Salmonella Set2-OrgC-Probe2
  misc_feature 6: note = n is inosine
  misc_feature 1..24: note = none, one or more, or each of nucleotides 9, 18, and 23 comprises 5-methylcytosine
  source 1..24: mol_type = other DNA
caggangtcatttgtgactgtgcg

SEQ ID NO: 27 - DNA, 25 bp, synthetic construct
  misc_feature 1..25: note = Synthetic: Salmonella Set3-InvA-RP
  misc_feature 1..25: note = none, one or more, or each of nucleotides 6, 10, and 18 comprises 5-methylcytosine
  source 1..25: mol_type = other DNA
cagtgcgatcaggaaatcaaccaga

SEQ ID NO: 28 - DNA, 27 bp, synthetic construct
  misc_feature 1..27: note = Synthetic: Salmonella Set1-InvA-RP
  misc_feature 18: note = n is inosine
  misc_feature 1..27: note = none, one or more, or each of nucleotides 2, 4, 12, 14, 15, and 17 comprises 5-methylcytosine
  source 1..27: mol_type = other DNA
ccacgaatatgctccacnaggttaatg

SEQ ID NO: 29 - DNA, 20 bp, synthetic construct
  misc_feature 1..20: note = Synthetic: Shigella Set1-ipaH-Probe2
  source 1..20: mol_type = other DNA
ccagagggagaaccagtccg

SEQ ID NO: 30 - DNA, 25 bp, synthetic construct
  misc_feature 1..25: note = Synthetic: Salmonella Set3-OrgC-Probe
  misc_feature 14: note = n is inosine
  misc_feature 23: note = n is inosine
  misc_feature 1..25: note = none, one or more, or each of nucleotides 2, 4, 18, 19, and 20 comprises 5-methylcytosine
  source 1..25: mol_type = other DNA
cctcatataaatgngtgcccggntc

SEQ ID NO: 31 - DNA, 27 bp, synthetic construct
  misc_feature 1..27: note = Synthetic: Salmonella Set2-InvA-RP
  misc_feature 20: note = n is inosine
  misc_feature 1..27: note = none, one or more, or each of nucleotides 6, 7, 8, 13, 23, 24, and 26 comprises 5-methylcytosine
  source 1..27: mol_type = other DNA
cggatccctttgcgaataanatcctca

SEQ ID NO: 32 - DNA, 22 bp, synthetic construct
  misc_feature 1..22: note = Synthetic: Shigella Set3-ipaH-FP
  misc_feature 9: note = n is inosine
  misc_feature 1..22: note = none, one or more, or each of nucleotides 5, 11, 12, and 15 comprises 5-methylcytosine
  source 1..22: mol_type = other DNA
cgggcaatntcctccagaattt

SEQ ID NO: 33 - DNA, 20 bp, synthetic construct
  misc_feature 1..20: note = Synthetic: Shigella Set3-ipaH-RP
  source 1..20: mol_type = other DNA
ctcctggtccatcaggcatc

SEQ ID NO: 34 - DNA, 21 bp, synthetic construct
  misc_feature 1..21: note = Synthetic: Shigella Set1-ipaH-FP
  source 1..21: mol_type = other DNA
cttccgtacgcttcagtacag

SEQ ID NO: 35 - DNA, 22 bp, synthetic construct
  misc_feature 1..22: note = Synthetic: Salmonella Set3-OrgC-FP
  source 1..22: mol_type = other DNA
gcagcaaacggctatgctacaa

SEQ ID NO: 36 - DNA, 25 bp, synthetic construct
  misc_feature 1..25: note = Synthetic: Salmonella Set2-OrgC-RP
  misc_feature 7: note = n is inosine
  misc_feature 1..25: note = none, one or more, or each of nucleotides 2, 3, 4, 16, 18, 19, and 22 comprises 5-methylcytosine
  source 1..25: mol_type = other DNA
gcccganaaaataatctcctgcatc

SEQ ID NO: 37 - DNA, 29 bp, synthetic construct
  misc_feature 1..29: note = Synthetic: C. coli Set1-cadF-Probe
  misc_feature 12: note = n is inosine
  misc_feature 1..29: note = none, one or more, or each of nucleotides 17, 22, 23, and 27 comprises 5-methylcytosine
  source 1..29: mol_type = other DNA
cggtgtagatanaagtcgtatccagacag

SEQ ID NO: 38 - DNA, 25 bp, synthetic construct
  misc_feature 1..25: note = Synthetic: Salmonella Set2-OrgC-FP
  misc_feature 22: note = n is inosine
  misc_feature 1..25: note = none, one or more, or each of nucleotides 4, 6, 7, and 8 comprises 5-methylcytosine
  source 1..25: mol_type = other DNA
gggcacccatttatatgaggcntta

SEQ ID NO: 39 - DNA, 26 bp, synthetic construct
  misc_feature 1..26: note = Synthetic: C. coli Set1-cadF-Probe2
  misc_feature 15: note = n is inosine
  misc_feature 1..26: note = none, one or more, or each of nucleotides 2, 9, 12, 19, 22, 24, and 25 comprises 5-methylcytosine
  source 1..26: mol_type = other DNA
tctggatacgacttntatctacaccg

SEQ ID NO: 40 - DNA, 23 bp, synthetic construct
  misc_feature 1..23: note = Synthetic: Salmonella Set3-OrgC-RP
  misc_feature 16: note = n is inosine
  misc_feature 19: note = n is inosine
  misc_feature 1..23: note = none, one or more, or each of nucleotides 4, 13, 18, and 22 comprises 5-methylcytosine
  source 1..23: mol_type = other DNA
ggtcatttgtgactgngcnttca

SEQ ID NO: 41 - DNA, 26 bp, synthetic construct
  misc_feature 1..26: note = Synthetic: Salmonella Set3-InvA-FP
  source 1..26: mol_type = other DNA
gtgctcgtttacgacctgaattactg

SEQ ID NO: 42 - DNA, 24 bp, synthetic construct
  misc_feature 1..24: note = Synthetic: Salmonella Set2-InvA-FP
  misc_feature 10: note = n is inosine
  misc_feature 16: note = n is inosine
  source 1..24: mol_type = other DNA
tcgtggagcnatggcncgttatat

SEQ ID NO: 43 - DNA, 27 bp, synthetic construct
  misc_feature 1..27: note = Synthetic: Salmonella Set3-InvA-Probe
  misc_feature 15: note = n is inosine
  misc_feature 1..27: note = none, one or more, or each of nucleotides 2, 9, 12, 16, 17, 22, 23, and 26 comprises 5-methylcytosine
  source 1..27: mol_type = other DNA
tctatgttcgtcatnccattacctacc

SEQ ID NO: 44 - DNA, 22 bp, synthetic construct
  misc_feature 1..22: note = Synthetic: Salmonella Set2-OrgC-Probe1
  misc_feature 5: note = n is inosine
  misc_feature 8: note = n is inosine
  misc_feature 1..22: note = none, one or more, or each of nucleotides 7, 9, 13, and 15 comprises 5-methylcytosine
  source 1..22: mol_type = other DNA
tgaangcncagtcacaaatgac

SEQ ID NO: 45 - DNA, 23 bp, synthetic construct
  misc_feature 1..23: note = Synthetic: Salmonella Set1-OrgC-Probe
  misc_feature 10: note = n is inosine
  misc_feature 15: note = n is inosine
  misc_feature 19: note = n is inosine
  misc_feature 1..23: note = none, one or more, or each of nucleotides 3, 6, 8, and 17 comprises 5-methylcytosine
  source 1..23: mol_type = other DNA
tgctgctcanaaganacanaagc

SEQ ID NO: 46 - DNA, 24 bp, synthetic construct
  misc_feature 1..24: note = Synthetic: Shigella Set1-ipaH-Probe1
  misc_feature 1..24: note = none, one or more, or each of nucleotides 5, 11, and 12 comprises 5-methylcytosine.
  source 1..24: mol_type = other DNA
tggtcagaagccgtgaagagaatg

SEQ ID NO: 47 - DNA, 20 bp, synthetic construct
  misc_feature 1..20: note = Synthetic: Salmonella Set1-OrgC-RP
  misc_feature 4: note = n is inosine
  misc_feature 1..20: note = none, one or more, or each of nucleotides 11, 16, and 17 comprises 5-methylcytosine
  source 1..20: mol_type = other DNA
tgtnttgtagcatagccgtt

SEQ ID NO: 48 - DNA, 25 bp, synthetic construct
  misc_feature 1..25: note = Synthetic: E. coli Set1-stx1-Probe
  source 1..25: mol_type = other DNA
acagcgtgttgcagggatcagtcgt

SEQ ID NO: 49 - DNA, 25 bp, synthetic construct
  misc_feature 1..25: note = Synthetic: E. coli Set1-stx1-FP
  source 1..25: mol_type = other DNA
cggttacattgtctggtgacagtag